European Patent Application EP 4 116 331 A1, published January 11, 2023. Title: Treatment of CD47+ Disease Cells with SIRP Alpha-Fc Fusions. Applicant: Trillium Therapeutics Inc. Application EP13865442.1. The sequence listing filed with the application follows.

SEQUENCE LISTING (28 sequences)

SEQ ID NO: 1 - protein, 106 aa, Homo sapiens
EELQVIQPDKSVSVAAGESAILHCTVTSLIPVGPIQWFRGAGPARELIYNQKEGHFPRVTTVSESTKRENMDFSISISNITPADAGTYYCVKFRKGSPDTEFKSGA

SEQ ID NO: 2 - protein, 227 aa, Homo sapiens
DKTHTCPPCPAPELLGGPSVFLFPPKPKDTLMISRTPEVTCVVVDVSHEDPEVKFNWYVDGVEVHNAKTKPREEQYNSTYRVVSVLTVLHQDWLNGKEYKCKVSNKALPAPIEKTISKAKGQPREPQVYTLPPSRDELTKNQVSLTCLVKGFYPSDIAVEWESNGQPENNYKTTPPVLDSDGSFFLYSKLTVDKSRWQQGNVFSCSVMHEALHNHYTQKSLSLSPGK

SEQ ID NO: 3 - protein, 345 aa, Homo sapiens
EEELQVIQPDKSVSVAAGESAILHCTVTSLIPVGPIQWFRGAGPARELIYNQKEGHFPRVTTVSESTKRENMDFSISISNITPADAGTYYCVKFRKGSPDTEFKSGAGTELSVRAKPSDKTHTCPPCPAPELLGGPSVFLFPPKPKDTLMISRTPEVTCVVVDVSHEDPEVKFNWYVDGVEVHNAKTKPREEQYNSTYRVVSVLTVLHQDWLNGKEYKCKVSNKALPAPIEKTISKAKGQPREPQVYTLPPSRDELTKNQVSLTCLVKGFYPSDIAVEWESNGQPENNYKTTPPVLDSDGSFFLYSKLTVDKSRWQQGNVFSCSVMHEALHNHYTQKSLSLSPGK

SEQ ID NO: 4 - protein, 375 aa, Homo sapiens
MEPAGPAPGRLGPLLCLLLAASCAWSGVAGEEELQVIQPDKSVSVAAGESAILHCTVTSLIPVGPIQWFRGAGPARELIYNQKEGHFPRVTTVSESTKRENMDFSISISNITPADAGTYYCVKFRKGSPDTEFKSGAGTELSVRAKPSDKTHTCPPCPAPELLGGPSVFLFPPKPKDTLMISRTPEVTCVVVDVSHEDPEVKFNWYVDGVEVHNAKTKPREEQYNSTYRVVSVLTVLHQDWLNGKEYKCKVSNKALPAPIEKTISKAKGQPREPQVYTLPPSRDELTKNQVSLTCLVKGFYPSDIAVEWESNGQPENNYKTTPPVLDSDGSFFLYSKLTVDKSRWQQGNVFSCSVMHEALHNHYTQKSLSLSPGK

SEQ ID NO: 5 - DNA, 318 bp, Homo sapiens
gaggagctgcaggtgattcagcctgacaagtccgtatcagttgcagctggagagtcggccattctgcactgcactgtgacctccctgatccctgtggggcccatccagtggttcagaggagctggaccagcccgggaattaatctacaatcaaaaagaaggccacttcccccgggtaacaactgtttcagagtccacaaagagagaaaacatggacttttccatcagcatcagtaacatcaccccagcagatgccggcacctactactgtgtgaagttccggaaagggagccctgacacggagtttaagtctggagca

SEQ ID NO: 6 - DNA, 684 bp, Homo sapiens
gacaaaactcacacatgcccaccgtgcccagcacctgaactcctggggggaccgtcagtcttcctcttcccaccaaaacccaaggacaccctcatgatctcccggacccctgaggtcacatgcgtggtggtggacgtgagccacgaagaccctgaggtcaagttcaactggtacgtggacggcgtggaggtgcataatgccaagacaaagccgcgggaggagcagtacaacagcacgtaccgtgtggtcagcgtcctcaccgtcctgcaccaggactggctgaatggcaaggagtacaagtgcaaggtctccaacaaagccctcccagcccccatcgagaaaaccatctccaaagccaaagggcagccccgagaaccacaggtgtacaccctgcccccatcccgggatgagctgaccaagaaccaggtcagcctgacctgcctggtcaaaggcttctatcccagcgacatcgccgtggagtgggagagcaatgggcagccggagaacaactacaagaccacgcctcccgtgctggactccgacggctccttcttcctctatagcaagctcaccgtggacaagagcaggtggcagcaggggaacgtcttctcatgctccgtgatgcatgaggctctgcacaaccactacacgcagaagagcctctccctgtctccgggtaaatga

SEQ ID NO: 7 - DNA, 1035 bp, Homo sapiens
gaggagctgcaggtgattcagcctgacaagtccgtatcagttgcagctggagagtcggccattctgcactgcactgtgacctccctgatccctgtggggcccatccagtggttcagaggagctggaccagcccgggaattaatctacaatcaaaaagaaggccacttcccccgggtaacaactgtttcagagtccacaaagagagaaaacatggacttttccatcagcatcagtaacatcaccccagcagatgccggcacctactactgtgtgaagttccggaaagggagccctgacacggagtttaagtctggagcaggcactgagctgtctgtgcgtgccaaaccctctgacaaaactcacacatgcccaccgtgcccagcacctgaactcctggggggaccgtcagtcttcctcttcccaccaaaacccaaggacaccctcatgatctcccggacccctgaggtcacatgcgtggtggtggacgtgagccacgaagaccctgaggtcaagttcaactggtacgtggacggcgtggaggtgcataatgccaagacaaagccgcgggaggagcagtacaacagcacgtaccgtgtggtcagcgtcctcaccgtcctgcaccaggactggctgaatggcaaggagtacaagtgcaaggtctccaacaaagccctcccagcccccatcgagaaaaccatctccaaagccaaagggcagccccgagaaccacaggtgtacaccctgcccccatcccgggatgagctgaccaagaaccaggtcagcctgacctgcctggtcaaaggcttctatcccagcgacatcgccgtggagtgggagagcaatgggcagccggagaacaactacaagaccacgcctcccgtgctggactccgacggctccttcttcctctatagcaagctcaccgtggacaagagcaggtggcagcaggggaacgtcttctcatgctccgtgatgcatgaggctctgcacaaccactacacgcagaagagcctctccctgtctccgggtaaatga

SEQ ID NO: 8 - DNA, 1128 bp, Homo sapiens
atggagcccgccggcccggcccccggccgcctcgggccgctgctctgcctgctgctcgccgcgtcctgcgcctggtcaggagtggcgggtgaggaggagctgcaggtgattcagcctgacaagtccgtatcagttgcagctggagagtcggccattctgcactgcactgtgacctccctgatccctgtggggcccatccagtggttcagaggagctggaccagcccgggaattaatctacaatcaaaaagaaggccacttcccccgggtaacaactgtttcagagtccacaaagagagaaaacatggacttttccatcagcatcagtaacatcaccccagcagatgccggcacctactactgtgtgaagttccggaaagggagccctgacacggagtttaagtctggagcaggcactgagctgtctgtgcgtgccaaaccctctgacaaaactcacacatgcccaccgtgcccagcacctgaactcctggggggaccgtcagtcttcctcttcccaccaaaacccaaggacaccctcatgatctcccggacccctgaggtcacatgcgtggtggtggacgtgagccacgaagaccctgaggtcaagttcaactggtacgtggacggcgtggaggtgcataatgccaagacaaagccgcgggaggagcagtacaacagcacgtaccgtgtggtcagcgtcctcaccgtcctgcaccaggactggctgaatggcaaggagtacaagtgcaaggtctccaacaaagccctcccagcccccatcgagaaaaccatctccaaagccaaagggcagccccgagaaccacaggtgtacaccctgcccccatcccgggatgagctgaccaagaaccaggtcagcctgacctgcctggtcaaaggcttctatcccagcgacatcgccgtggagtgggagagcaatgggcagccggagaacaactacaagaccacgcctcccgtgctggactccgacggctccttcttcctctatagcaagctcaccgtggacaagagcaggtggcagcaggggaacgtcttctcatgctccgtgatgcatgaggctctgcacaaccactacacgcagaagagcctctccctgtctccgggtaaatga

SEQ ID NO: 9 - DNA, 20 bp, Artificial Sequence
  primer
ggcgctagccaccatggagc

SEQ ID NO: 10 - DNA, 21 bp, Artificial Sequence
  primer
ggtgaagctcactgtgtgctg

SEQ ID NO: 11 - DNA, 21 bp, Artificial Sequence
  primer
cagcacacagtgagcttcacc

SEQ ID NO: 12 - DNA, 20 bp, Artificial Sequence
  primer
ccggatcctcatttacccag

SEQ ID NO: 13 - DNA, 27 bp, Artificial Sequence
  primer
ggactcagagggtttggcacgcacaga

SEQ ID NO: 14 - DNA, 27 bp, Artificial Sequence
  primer
ccctctgagtccaaatatggtccccca

SEQ ID NO: 15 - DNA, 30 bp, Artificial Sequence
  primer
agttttgtcagagggtttggcacgcacaga

SEQ ID NO: 16 - DNA, 30 bp, Artificial Sequence
  primer
aaaccctctgacaaaactcacacatgccca

SEQ ID NO: 17 - DNA, 21 bp, Artificial Sequence
  primer
cacggatcctcatttacccgg

SEQ ID NO: 18 - DNA, 27 bp, Artificial Sequence
  primer
aggtgctgggcatggtgggcatggggg

SEQ ID NO: 19 - DNA, 27 bp, Artificial Sequence
  primer
cccccatgcccaccatgcccagcacct

SEQ ID NO: 20 - DNA, 29 bp, Artificial Sequence
  primer
cacggatcctcatttacccagagacaggg

SEQ ID NO: 21 - protein, 11 aa, Artificial Sequence
  amino acid linker
GTELSVRAKPS

SEQ ID NO: 22 - protein, 118 aa, Homo sapiens
EEELQVIQPDKSVSVAAGESAILHCTVTSLIPVGPIQWFRGAGPARELIYNQKEGHFPRVTTVSESTKRENMDFSISISNITPADAGTYYCVKFRKGSPDTEFKSGAGTELSVRAKPS

SEQ ID NO: 23 - protein, 229 aa, Homo sapiens
ESKYGPPCPSCPAPEFLGGPSVFLFPPKPKDTLMISRTPEVTCVVVDVSQEDPEVQFNWYVDGVEVHNAKTKPREEQFNSTYRVVSVLTVLHQDWLNGKEYKCKVSNKGLPSSIEKTISKAKGQPREPQVYTLPPSQEEMTKNQVSLTCLVKGFYPSDIAVEWESNGQPENNYKTTPPVLDSDGSFFLYSRLTVDKSRWQEGNVFSCSVMHEALHNHYTQKSLSLSLGK

SEQ ID NO: 24 - protein, 229 aa, Homo sapiens
ESKYGPPCPPCPAPEFLGGPSVFLFPPKPKDTLMISRTPEVTCVVVDVSQEDPEVQFNWYVDGVEVHNAKTKPREEQFNSTYRVVSVLTVLHQDWLNGKEYKCKVSNKGLPSSIEKTISKAKGQPREPQVYTLPPSQEEMTKNQVSLTCLVKGFYPSDIAVEWESNGQPENNYKTTPPVLDSDGSFFLYSRLTVDKSRWQEGNVFSCSVMHEALHNHYTQKSLSLSLGK

SEQ ID NO: 25 - protein, 345 aa, Homo sapiens; identical to SEQ ID NO: 3

SEQ ID NO: 26 - protein, 347 aa, Homo sapiens
EEELQVIQPDKSVSVAAGESAILHCTVTSLIPVGPIQWFRGAGPARELIYNQKEGHFPRVTTVSESTKRENMDFSISISNITPADAGTYYCVKFRKGSPDTEFKSGAGTELSVRAKPSESKYGPPCPPCPAPEFLGGPSVFLFPPKPKDTLMISRTPEVTCVVVDVSQEDPEVQFNWYVDGVEVHNAKTKPREEQFNSTYRVVSVLTVLHQDWLNGKEYKCKVSNKGLPSSIEKTISKAKGQPREPQVYTLPPSQEEMTKNQVSLTCLVKGFYPSDIAVEWESNGQPENNYKTTPPVLDSDGSFFLYSRLTVDKSRWQEGNVFSCSVMHEALHNHYTQKSLSLSLGK

SEQ ID NO: 27 - DNA, 1128 bp, Homo sapiens; identical to SEQ ID NO: 8

SEQ ID NO: 28 - DNA, 1134 bp, Homo sapiens
atggagcccgccggcccggcccccggccgcctcgggccgctgctctgcctgctgctcgccgcgtcctgcgcctggtcaggagtggcgggtgaggaggagctgcaggtgattcagcctgacaagtccgtatcagttgcagctggagagtcggccattctgcactgcactgtgacctccctgatccctgtggggcccatccagtggttcagaggagctggaccagcccgggaattaatctacaatcaaaaagaaggccacttcccccgggtaacaactgtttcagagtccacaaagagagaaaacatggacttttccatcagcatcagtaacatcaccccagcagatgccggcacctactactgtgtgaagttccggaaagggagccctgacacggagtttaagtctggagcaggcactgagctgtctgtgcgtgccaaaccctctgagtccaaatatggtcccccatgcccaccatgcccagcacctgagttcctggggggaccatcagtcttcctgttccccccaaaacccaaggacactctcatgatctcccggacccctgaggtcacgtgcgtggtggtggacgtgagccaggaagaccccgaggtccagttcaactggtacgtggatggcgtggaggtgcataatgccaagacaaagccgcgggaggagcagttcaacagcacgtaccgtgtggtcagcgtcctcaccgtcctgcaccaggactggctgaacggcaaggagtacaagtgcaaggtctccaacaaaggcctcccgtcctccatcgagaaaaccatctccaaagccaaagggcagccccgagagccacaggtgtacaccctgcccccatcccaggaggagatgaccaagaaccaggtcagcctgacctgcctggtcaagggcttctaccccagcgacatcgccgtggagtgggagagcaatgggcagccggagaacaactacaagaccacgcctcccgtgctggactccgacggctccttcttcctctacagcaggctaaccgtggacaagagcaggtggcaggaggggaatgtcttctcatgctccgtgatgcatgaggctctgcacaaccactacacgcagaagagcctctccctgtctctgggtaaatga